European Patent Specification EP 3 411 066 B1, published May 13, 2026. Title: PARATHYROID HORMONE - ANTI-RANKL ANTIBODY FUSION COMPOUNDS. Applicant: ELI LILLY AND COMPANY. The sequence listing filed with the application follows.

SEQUENCE LISTING (15 sequences)

SEQ ID NO: 1 - protein, 496 aa, Artificial Sequence
  Exemplified First Polypeptide (of exemplified fusion compound of Table 1)
SVSEIQLMHNLGKHLNSMERVEWLRKKLQDVHNFGGGGSGGGGSGGGGSQVQLVQSGAEVKKPGSSVKVSCKASGYAFTNYYIEWVRQAPGQGLEWMGVINPGWGDTNYNEKFKGRVTITADKSTSTAYMELSSLRSEDTAVYYCARRDTAHGYYALDPWGQGTTVTVSSASTKGPSVFPLAPCSRSTSESTAALGCLVKDYFPEPVTVSWNSGALTSGVHTFPAVLQSSGLYSLSSVVTVPSSSLGTKTYTCNVDHKPSNTKVDKRVESKYGPPCPPCPAPEAAGGPSVFLFPPKPKDTLMISRTPEVTCVVVDVSQEDPEVQFNWYVDGVEVHNAKTKPREEQFNSTYRVVSVLTVLHQDWLNGKEYKCKVSNKGLPSSIEKTISKAKGQPREPQVYTLPPSQEEMTKNQVSLTCLVKGFYPSDIAVEWESNGQPENNYKTTPPVLDSDGSFFLYSRLTVDKSRWQEGNVFSCSVMHEALHNHYTQKSLSLSLG

SEQ ID NO: 2 - protein, 214 aa, Artificial Sequence
  Exemplified Second Polypeptide (of the exemplified fusion compound of Table 1)
DIQMTQSPSSLSASVGDRVTITCKASQNVGTNVAWYQQKPGKAPKLLIYSASYRYSGVPSRFSGSGSGTDFTLTISSLQPEDFATYYCQQYWDYPLTFGGGTKVEIKRTVAAPSVFIFPPSDEQLKSGTASVVCLLNNFYPREAKVQWKVDNALQSGNSQESVTEQDSKDSTYSLSSTLTLSKADYEKHKVYACEVTHQGLSSPVTKSFNRGEC

SEQ ID NO: 3 - DNA, 1491 bp, Artificial Sequence
  DNA Seq. Encoding the Exemplified First Polypeptide (SEQ ID NO. 1) and a Signal Peptide
agcgtgtccgagatccagctgatgcacaacctcggcaagcacctgaatagcatggagcgcgtcgagtggctgcggaagaaactgcaggacgtgcacaacttcggcggcggcggcagcggcggtggcggctccggtggcggcggaagccaggtgcagctggtgcagtctggggctgaggtgaagaagcctgggtcctcagtgaaggtttcctgcaaggcatctggctacgccttcaccaactactatatcgagtgggtgcgacaggcccctggacaagggcttgagtggatgggagtgatcaaccccggctggggcgacacgaactacaacgagaagttcaagggcagagtcaccattaccgcggacaaatccacgagcacagcctacatggagctgagcagcctgagatctgaggacacggccgtgtattactgtgcgagacgcgatacggctcacggctactacgcccttgatccgtggggccaaggaaccacggtcaccgtctcctcagcctccaccaagggcccatcggtcttcccgctagcgccctgctccaggagcacctccgagagcacagccgccctgggctgcctggtcaaggactacttccccgaaccggtgacggtgtcgtggaactcaggcgccctgaccagcggcgtgcacaccttcccggctgtcctacagtcctcaggactctactccctcagcagcgtggtgaccgtgccctccagcagcttgggcacgaagacctacacctgcaacgtagatcacaagcccagcaacaccaaggtggacaagagagttgagtccaaatatggtcccccatgcccaccctgcccagcacctgaggccgccgggggaccatcagtcttcctgttccccccaaaacccaaggacactctcatgatctcccggacccctgaggtcacgtgcgtggtggtggacgtgagccaggaagaccccgaggtccagttcaactggtacgtggatggcgtggaggtgcataatgccaagacaaagccgcgggaggagcagttcaacagcacgtaccgtgtggtcagcgtcctcaccgtcctgcaccaggactggctgaacggcaaggagtacaagtgcaaggtctccaacaaaggcctcccgtcctccatcgagaaaaccatctccaaagccaaagggcagccccgagagccacaggtgtacaccctgcccccatcccaggaggagatgaccaagaaccaggtcagcctgacctgcctggtcaaaggcttctaccccagcgacatcgccgtggagtgggaaagcaatgggcagccggagaacaactacaagaccacgcctcccgtgctggactccgacggctccttcttcctctacagcaggctaaccgtggacaagagcaggtggcaggaggggaatgtcttctcatgctccgtgatgcatgaggctctgcacaaccactacacacagaagagcctctccctgtctctgggttga

SEQ ID NO: 4 - DNA, 690 bp, Artificial Sequence
  DNA Seq. Encoding the Exemplified Second Polypeptide (SEQ ID NO. 2) and a Signal Peptide
ggcggcggcggcagcggcggtggcggctccggtggcggcggaagcgacatccagatgacccagtctccatcctctctgtctgcatctgtaggagacagagtcaccatcacttgcaaggccagccagaatgtgggcaccaacgtggcctggtatcagcagaaaccagggaaagcccctaagctcctgatctatagcgccagctacagatacagcggggtcccatcaaggttcagtggcagtggatctgggacagatttcactctcaccatcagcagtctgcaacctgaagattttgcaacttactactgtcagcagtactgggactaccccctgaccttcggcggagggaccaaggtggagatcaaacggactgtggctgcaccatctgtcttcatcttcccgccatctgatgagcagttgaaatctggaactgcctctgttgtgtgcctgctgaataacttctatcccagagaggccaaagtacagtggaaggtggataacgccctccaatcgggtaactcccaggagagtgtcacagagcaggacagcaaggacagcacctacagcctcagcagcaccctgacgctgagcaaagcagactacgagaaacacaaagtctacgcctgcgaagtcacccatcagggcctgagctcgcccgtcacaaagagcttcaacaggggagagtgctaa

SEQ ID NO: 5 - protein, 121 aa, Artificial Sequence
  Exemplified HCVR (of exemplified fusion compound of Table 1)
QVQLVQSGAEVKKPGSSVKVSCKASGYAFTNYYIEWVRQAPGQGLEWMGVINPGWGDTNYNEKFKGRVTITADKSTSTAYMELSSLRSEDTAVYYCARRDTAHGYYALDPWGQGTTVTVSS

SEQ ID NO: 6 - protein, 107 aa, Artificial Sequence
  Exemplified LCVR (of exemplified fusion compound of Table 1)
DIQMTQSPSSLSASVGDRVTITCKASQNVGTNVAWYQQKPGKAPKLLIYSASYRYSGVPSRFSGSGSGTDFTLTISSLQPEDFATYYCQQYWDYPLTFGGGTKVEIK

SEQ ID NO: 7 - protein, 10 aa, Artificial Sequence
  Exemplified HCDR1 (of exemplified fusion compound of Table 1)
GYAFTNYYIE

SEQ ID NO: 8 - protein, 17 aa, Artificial Sequence
  Exemplified HCDR2 (of exemplified fusion compound of Table 1)
VINPGWGDTNYNEKFKG

SEQ ID NO: 9 - protein, 12 aa, Artificial Sequence
  Exemplified HCDR3 (of exemplified fusion compound of Table 1)
RDTAHGYYALDP

SEQ ID NO: 10 - protein, 11 aa, Artificial Sequence
  Exemplified LCDR1 (of exemplified fusion compound of Table 1)
KASQNVGTNVA

SEQ ID NO: 11 - protein, 7 aa, Artificial Sequence
  Exemplified LCDR2 (of exemplified fusion compound of Table 1)
SASYRYS

SEQ ID NO: 12 - protein, 9 aa, Artificial Sequence
  Exemplified LCDR3 (of exemplified fusion compound of Table 1)
QQYWDYPLT

SEQ ID NO: 13 - protein, 34 aa, Artificial Sequence
  Exemplified PTH Peptide of exemplified fusion compound of Table 1
SVSEIQLMHNLGKHLNSMERVEWLRKKLQDVHNF

SEQ ID NO: 14 - protein, 15 aa, Artificial Sequence
  Exemplified Linker of exemplified fusion compound of Table 1
GGGGSGGGGSGGGGS

SEQ ID NO: 15 - protein, 84 aa, Artificial Sequence
  Full length Human Parathyroid Hormone
SVSEIQLMHNLGKHLNSMERVEWLRKKLQDVHNFVALGAPLAPRDAGSQRPRKKEDNVLVESHEKSLGEADKADVNVLTKAKSQ